European Patent Application EP 4 495 243 A1, published January 22, 2025. Title: Novel method for producing exosomes loaded with nucleic acids of interest. Applicant: PROGENICYTE JAPAN CO.,LTD. The sequence listing filed with the application follows.

SEQUENCE LISTING (9 sequences)

SEQ ID NO: 1 - DNA, 22 bp, Homo sapiens
  source 1..22: mol_type = genomic DNA
gctaaggacaacattgatagaa

SEQ ID NO: 2 - DNA, 27 bp, synthetic construct
  misc_feature 1..27: note = primer
  source 1..27: mol_type = other DNA
atatggatccggatggtctcgatctcc

SEQ ID NO: 3 - DNA, 17 bp, synthetic construct
  misc_feature 1..17: note = primer
  source 1..17: mol_type = other DNA
gggactagtcctgcagg

SEQ ID NO: 4 - DNA, 17 bp, synthetic construct
  misc_feature 1..17: note = primer
  source 1..17: mol_type = other DNA
accacgatgcctgtagc

SEQ ID NO: 5 - DNA, 17 bp, synthetic construct
  misc_feature 1..17: note = primer
  source 1..17: mol_type = other DNA
gcgcagaagtggtcctg

SEQ ID NO: 6 - DNA, 17 bp, synthetic construct
  misc_feature 1..17: note = primer
  source 1..17: mol_type = other DNA
gtgctcgacgttgtcac

SEQ ID NO: 7 - DNA, 17 bp, synthetic construct
  misc_feature 1..17: note = primer
  source 1..17: mol_type = other DNA
ccggatcaagcgtatgc

SEQ ID NO: 8 - DNA, 20 bp, synthetic construct
  source 1..20: mol_type = other DNA
gtgggaggttttttaaagca

SEQ ID NO: 9 - DNA, 20 bp, synthetic construct
  source 1..20: mol_type = other DNA
acagacaatcggctgctctg